European Patent Specification EP 3 908 680 B1, published March 1, 2023. Title: METHODS FOR SCREENING INHIBITORS AGAINST CHIKUNGUNYA VIRUS AND FOR DETERMINING WHETHER SUBJECTS ARE PREDISPOSED TO INFECTION BY SAID VIRUS. Applicant: Inserm. The sequence listing filed with the application follows.

SEQUENCE LISTING (4 sequences)

SEQ ID NO: 1 - protein, 279 aa, Homo sapiens
AEKFDCHYCRDPLQGKKYVQKDGHHCCLKCFDKFCANTCVECRKPIGADSKEVHYKNRFWHDTCFRCAKCLHPLANETFVAKDNKILCNKCTTREDSPKCKGCFKAIVAGDQNVEYKGTVWHKDCFTCSNCKQVIGTGSFFPKGEDFYCVTCHETKFAKHCVKCNKAITSGGITYQDQPWHADCFVCVTCSKKLAGQRFTAVEDQYYCVDCYKNFVAKKCAGCKNPITGFGKGSSVVAYEGQSWHDYCFHCKKCSVNLANKRFVFHQEQVYCPDCAKKL

SEQ ID NO: 2 - protein, 323 aa, Homo sapiens
MAEKFDCHYCRDPLQGKKYVQKDGHHCCLKCFDKFCANTCVECRKPIGADSKEVHYKNRFWHDTCFRCAKCLHPLANETFVAKDNKILCNKCTTREDSPKCKGCFKAIVAGDQNVEYKGTVWHKDCFTCSNCKQVIGTGSFFPKGEDFYCVTCHETKFAKHCVKCNKAITSGGITYQDQPWHADCFVCVTCSKKLAGQRFTAVEDQYYCVDCYKNFVAKKCAGCKNPITGKRTVSRVSHPVSKARKPPVCHGKRLPLTLFPSANLRGRHPGGERTCPSWVVVLYRKNRSLAAPRGPGLVKAPVWWPMKDNPGTTTASTAKNAP

SEQ ID NO: 3 - protein, 194 aa, Homo sapiens
MAEKFDCHYCRDPLQGKKYVQKDGHHCCLKCFDKFCANTCVECRKPIGADSKEVHYKNRFWHDTCFRCAKCLHPLANETFVAKDNKILCNKCTTREDSPKCKGCFKAIVAGDQNVEYKGTVWHKDCFTCSNCKQVIGTGSFFPKGEDFYCVTCHETKFAKHCVKCNKGLVKAPVWWPMKDNPGTTTASTAKNAP

SEQ ID NO: 4 - protein, 524 aa, Chikungunya virus
MAPSYRVKRMDIAKNDEECVVNAANPRGLPGDGVCKAVYKKWPESFKNSATPVGTAKTVMCGTYPVIHAVGPNFSNYSESEGDRELAAAYREVAKEVTRLGVNSVAIPLLSTGVYSGGKDRLTQSLNHLFTAMDSTDADVVIYCRDKEWEKKISEAIQMRTQVELLDEHISIDCDIVRVHPDSSLAGRKGYSTTEGALYSYLEGTRFHQTAVDMAEIHTMWPKQTEANEQVCLYALGESIESIRQKCPVDDADASSPPKTVPCLCRYAMTPERVTRLRMNHVTSIIVCSSFPLPKYKIEGVQKVKCSKVMLFDHNVPSRVSPREYRSSQESAQEASTITSLTHSQFDLSVDGEILPVPSDLDADAPALEPALDDGATHTLPSTTGNLAAVSDWVISTVPVAPPRRRRGRNLTVTCDEREGNITPMASVRFFRAELCPVVQETAETRDTAMSLQAPPSTATEPNHPPISFGASSETFPITFGDFNEGEIESLSSELLTFGDFLPGEVDDLTDSDWSTCSDTDDEL